European Patent Application EP 4 772 628 A1, published July 8, 2026. Title: 非天然RNA 的制备方法及产品. Applicant: 吉林凯莱英医药化学有限公司. The sequence listing filed with the application follows.

SEQUENCE LISTING (30 sequences)

SEQ ID NO: 1 - protein, 334 aa, Bacteriophage
MFKKYSSLENHYNSKFIEKLYSLGLTGGEWVAREKIHGTNFSLIIERDKVTCAKRTGPILPAEDFFGYEIILKNYADSIKAVQDIMETSAVVSYQVFGEFAGPGIQKNVDYCDKDFYVFDIIVTTESGDVTYVDDYMMESFCNTFKFKMAPLLGRGKFEELIKLPNDLDSVVQDYNFTVDHAGLVDANKCVWNAEAKGEVFTAEGYVLKPCYPSWLRNGNRVAIKCKNSKFSEKKKSDKPIKAKVELSEADNKLVGILACYVTLNRVNNVISKIGEIGPKDFGKVMGLTVQDILEETSREGITLTQADNPSLIKKELVKMVQDVLRPAWIELVS

SEQ ID NO: 2 - protein, 335 aa, Vibrio phage
MSFVKYTSLENSYRQAFVDKCDMLGVREWVALEKIHGANFSFIVEFKPNEAQDGAEFTVTPAKRTSTIGANVMGDYDFYGCTSVVEAHTAKMEAISNWLWARGIINVGETIIVYGELAGKGVQKEVNYGDKDFWAYDILLPETGKFLDWDVVLEACEFAKVKTTHEIARGTLDELLRIDPLFRSFHTPADVDGDNVAEGFVVKQLRNEKRLHNGSRAILKVKNDKFKEKKNKAGKTPRAAVVLTEEQEKLHAAFSCYLTENRLRNVLSKLETVTQKQFGMISGLFIKDAKDEFERDELNETAIARDDWDVIKRSLTNIANEILRKNWLDILDGNF

SEQ ID NO: 3 - protein, 374 aa, Bacteriophage AR1
MQELFNNLMELCKDSQRKFFYSDDVSASGRTYRIFSYNYASYSDWLLPDALECRGIMFEMDGEKPVRIASRPMEKFFNLNENPFTMNIDLNDVDYILTKEDGSLVSTYLDGDEILFKSKGSIKSEQALMANGILMNINHHQLRDRLKELAEDGFTANFEFVAPTNRIVLAYQEMKIILLNIRENETGEYISYDDIYKDAALRPYLVERYEIDSPKWVEEAKNAENIEGYVAVMKDGSHFKIKSDWYVSLHSTKSSLDNPEKLFKTIIDGASDDLKAMYADDEYSYRKIEAFETTYLKYLDRALFLVLDCHNKHCGKDRKTYAMEAQGVAKGAGMDHLFGIIMSLYQGYDSQEKVMCEIEQNFLKNYKKFIPEGY

SEQ ID NO: 4 - protein, 335 aa, Bacteriophage dhaeg
MFKKYSSLENHYNSKFIEKLRTNGLTGGEWVAREKIHGTNFSLIIERDAVTCAKRTGPILPAEDFYGYEIVLKNYADSIKSIQDIMETSAAVSYQVFGEFAGTGIQKNVDYGDKDFYVFDIIVTTESGDVTYVDDYMMESFCKTFKFKMAPLLGRGKFEDLIKLPNDLDSVLPDYNFTVDNVGLAEANAHVWNAEAKGEVFTAEGYVLKPCYPLWLPNGNRVAIKCKNSKFSEKKKTDKPIKVAVVLSQDDLDLLQQFTDYVTVNRINNVISKIGEVSPKDFGKVMGLTVQDILEEAAREELELTDAENPVEVKKQLIECVKDTLRAVWIELVSK

SEQ ID NO: 5 - protein, 383 aa, Klebsiella phage KP179
MLELYKNLMNLCESSEVAKFFYKDFTGPMDGKFRVFSYHYASYSEWLKPDALECRGIMFEMDGDTPIRIASRPMEKFFNLNENPLTMGIDISDVEYIMDKADGSLVSSYVDDGYLYLKSKTSLYSDQARQASALLNSEEYSSLHQVILELTLDGYTVNMEFVSPNNRVVLAYQEPQLFVLNVRNNTTGEYIKYDDLYANAKIRPYLINAYGISDPTTWVEGVRELEGVEGYIAVLNTGQRFKVKTEWYSALHHTKDSITSNERLFASVVSANSDDLRSLFAGDEYAIKKISAFEQAYLDYLGKSLELCQSFYDEYRGRARKDYAIAAQKATVNQRHLFGVIMNMYEGTVDVDKLLKDLERVFLKYWAGYVPKEYEKEIELSEE

SEQ ID NO: 6 - protein, 381 aa, Vibrio phage
MTTQELYNHLMTLTDDAEGKFFFADHISPLGEKLRVFSYHIASYSDWLLPGALEARGIMFQLDEQDKMVRIVSRPMEKFFNLNENPFTMDLDLTTTVQLMDKADGSLISTYLTGENFALKSKTSIFSEQAVAANRYIKLPENRDLWEFCDDLTQAGCTVNMEWCAPNNRIVLEYPEAKLVILNIRDNETGDYVSFDDIPLPALMRVKKWLVDEYDPETAHADDFVEKLRATKGIEGMILRLANGQSVKIKTQWYVDLHSQKDSVNVPKKLVTTILNNNHDDLYALFADDKPTIDRIREFDSHVSKTVSASFHAVSQFYVKNRHMSRKDYAIAGQKTLKPWEFGVAMIAYQNQTVEGVYEALVGAYLKRPELLIPEKYLNEA

SEQ ID NO: 7 - protein, 374 aa, Escherichia phage JN02
MEKLYYNLLSLCKSSSDRKFFYSDDVSPIGKKYRIFSYNFASYSDWLLPDALECRGIMFEMDGETPVRIASRPMEKFFNLNENPFTLSINLDDVKYLMTKEDGSLVSTYLDGGTVRFKSKGSIKSDQAVSATSILLDIDHKNLADRLLELCNDGFTANFEYVAPTNKIVLTYPEKRLILLNIRDNNTGEYIEYDDIYLDPVFRKYLVDRFEVPEGDWTSDVKSSTNIEGYVAVMKDGSHFKLKTDWYVALHTTRDSISSPEKLFLAIVNGASDDLKAMYADDEFSFKKVELFEKAYLDFLDRSFYICLDTYDKHKGKDRKTYAIEAQAVCKGAQTPWLFGIIMNLYQGGSKEQMMTALESVFIKNHKNFIPEGY

SEQ ID NO: 8 - protein, 339 aa, Klebsiella phage KP15
MFKKYSSLTNHYEGKFINGVIMNGLTGGVWVAREKIHGANFSFITDDGITVTPAKRTDVVKPAEDFYGCSAVVAKYSPGIRKMWETLKKTGTYDDLVIQVYGEFAGRGVQKDVDYGEKDFYVFDIRVNGEFLPDNLCSLISRSHGLKMAPLLGYGTFEEIKELPITFESVVNKANSGIGSDNTVYGEFVYPIMDVEEGNIAEGFVMKPVSPAFMPNGERVAIKCKTTKFTEKKAKKATRFNAPVSLSEKDKNQLDEFVCYLTENRVKNVLSKLDLASITAKDFGRIMGLTVQDAIEEISRNHGPFIEQFEDPAMAKKLFVTEAQNMIRPVWGKILNHEF

SEQ ID NO: 9 - protein, 380 aa, Thermococcus
MVSSYFRNLLLKLGLPEERLEVLEGKGALAEDEFEGIRYVRFRDSARNFRRGTVVFETGEAVLGFPHIKRVVQLENGIRRVFKNKPFYVEEKVDGYNVRVVKVKDKILAITRGGFVCPFTTERIEDFVNFDFFKDYPNLVLVGEMAGPESPYLVEGPPYVKEDIEFFLFDIQEKGTGRSLPAEERYRLAEEYGIPQVERFGLYDSSKVGELKELIEWLSEEKREGIVMKSPDMRRIAKYVTPYANINDIKIGSHIFFDLPHGYFMGRIKRLAFYLAENHVRGEEFENYAKALGTALLRPFVESIHEVANGGEVDETFTVRVKNITTAHKMVTHFERLGVKIHIEDIEDLGNGYWRITFKRVYPDATREIRELWNGLAFVD

SEQ ID NO: 10 - protein, 487 aa, Archaea
MVVPLKRIDKIRWEIPKFDKRMRVPGRVYADEVLLEKMKNDRTLEQATNVAMLPGIYKYSIVMPDGHQGYGFPIGGVAAFDVKEGVISPGGIGYDINCGVRLIRTNLTEKEVRPRIKQLVDTLFKNVPSGVGSQGRIKLHWTQIDDVLVDGAKWAVDNGYGWERDLERLEEGGRMEGADPEAVSQRAKQRGAPQLGSLGSGNHFLEVQVVDKIFDPEVAKAYGLFEGQVVVMVHTGSRGLGHQVASDYLRIMERAIRKYRIPWPDRELVSVPFQSEEGQRYFSAMKAAANFAWANRQMITHWVRESFQEVFKQDPEGDLGMDIVYDVAHNIGKVEEHEVDGKRVKVIVHRKGATRAFPPGHEAVPRLYRDVGQPVLIPGSMGTASYILAGTEGAMKETFGSTCHGAGRVLSRKAATRQYRGDRIRQELLNRGIYVRAASMRVVAEEAPGAYKNVDNVVKVVSEAGIAKLVARMRPIGVAKGAAALEH

SEQ ID NO: 11 - protein, 438 aa, thermophilic bacteriophage
MESMNVKYPVEYLIEHLNSFESPEVAVESLRKEGIMCKNRGDLYMFKYHLGCKFDKIYHLACRGAILRKTDSGWKVLSYPFDKFFNWGEELQPEIVNYYQTLRYASPLNEKRKAGFMFKLPMKLVEKLDGTCVVLYYDEGWKIHTLGSIDANGSIVKNGMVTTHMDKTYRELFWETFEKKYPPYLLYHLNSSYCYIFEMVHPDARVVVPYEEPNIILIGVRSVDPEKGYFEVGPSEEAVRIFNESGGKINLKLPAVLSQEQNYTLFRANRLQELFEEVTPLFKSLRDGYEVVYEGFVAVQEIAPRVYYRTKIKHPVYLELHRIKTTITPEKLADLFLENKLDDFVLTPDEQETVMKLKEIYTDMRNQLESSFDTIYKEISEQVSPEENPGEFRKRFALRLMDYHDKSWFFARLDGDEEKMQKSEKKLLTERIEKGLFK

SEQ ID NO: 12 - protein, 203 aa, Diplonema papillatum
MPLSQGAALIRSPTVTAEEKVDGSNLAVYLDASGAVTCQNRGKFVTPSSGSQWGGQLATWLESHYCELVSLLRQRYILYGEWLLARHSIRYQSLPDYFVAFDVYDRTARRFLSAKKRNAFLSQSTIPVVKPLAVGPFAEADILRLLGSPSRYGAAKVEGIYLRSDSGAWLQQRAKVVNSDFLQTIDDDGHWQKRVLEKNQLKY

SEQ ID NO: 13 - protein, 553 aa, virus
MVYICIDTGSHAKGYAVESSDTDYHIYTKCDRETFEKFIDNKELLKNRHAKDESGNDVKYVDLYTGLIGILTGKSPELSMFSKREDFKDKYGIENLQLYEFVTKLMTVSMVKIIYTLMRYKILNNAKGLLQLMFNYVYVEYYLDYKRAPKSTKILNMLFNVGDEIKITMDKNNQLVVNDLNVLDLNKNNGGYKIDETLTLFVKNVKLLKLYVKLMQRGEYQQEWTEYFQQWKQQLQDRLHHVPEPPERTDIRHNIVMYALNERGPVMPEDENKIVYQIYPSVSHLDQGKKGTLADKEIIVQEKLDGCNFRIICNQNKITYGSRNTYRPDGNFMNYYRIRKDLETCMRSLQARFNDGFIVYGELMGWKDDAKTTPINVINYVDQKESLKYYAYEIQLYGGEFVPFVEAQELLTNVGFNTIPCHKYLYNDFVERLNFKSLMFPQSPLEGFIIRCGNLIYKLKSDYKDLNKLKIEKGPFEWLTCDYIKSNCDAIDKSDMMKILIFCYNMCKVKNYNEKLLFNKVFNLFRQQFNLNHNDYKNLYKQYVNMCKCTEYK

SEQ ID NO: 14 - protein, 379 aa, Archaea
MVSSVYKEILVKLGLTEDRIETLEMKGGIIEDEFDGIRYVRFKDSAGKLRRGTVVIDEEYVIPGFPHIKRIINLRSGIRRIFKRGEFYVEEKVDGYNVRVVMYKGKMLGITRGGFICPFTTERIPDFVPQEFFKDNPNLILVGEMAGPESPYLVEGPPYVKEDIQFFLFDVQEIKTGRSLPVEERLKIAEEYGINHVEVFGKYTKDDVDELYQLIERLSKEGREGIIMKSPDMKKIVKYVTPYANINDIKIGARVFYELPPGYFTSRISRLAFYLAEKRIKGEEFERVAKELGSALLQPFVESIFDVEQEEDIHELFKVRVKRIETAYKMVTHFEKLGLKIEIVDIEEIKDGWRITFKRLYPDATNEIRELIGGKAFVD

SEQ ID NO: 15 - protein, 416 aa, Trypanosoma brucei gambiense
MLRCLGVRHFRRTPLLFVGGDGSIFERYTEIDNSNERRINALKGCGMFEDEWIATEKVHGANFGIYSIEGEKMIRYAKRSGIMPPNEHFFGYHILIPELQRYVTSIREMLCEKQKKKLHVVLINGELFGGKYDHPSVPKTRKTVMVAGKPRTISAVQTDSFPQYSPDLHFYAFDIKYKETEGGDYTTLVYDEAIELFQRVPGLLYARAVIRGPMSKVAAFDVERFVTTIPPLVGMGNYPLTGNWAEGLVVKHSRLGMAGFDPKGPTVLKFKCTAFQEISTDRAQGPRVDEMRNVRRDSINRAGVQLPDLESIVQDPIQLEASKLLLNHVCENRLKNVLSKIGTEPFEKEEMTPDQLATLLAKDAMKDFLKDTEPSIVNIPVLIRKDLTRYVIFESRRLVCSQWKDILKRQSPDFSE

SEQ ID NO: 16 - protein, 382 aa, Acidobacteria bacterium
MKQMYDNLKALTQKNDMFFSSIQTTPSNKPVEIFSYHIASYSDWLEPDAIECRGIMFDITDKENPVILSRPMEKFFNLGENPLALPEDVLPLVKTIEEKRDGSLISTYLDDGKLYTKSKGSLYSDQANDSNRFLMRSENKDFKQALKTLAELGYTANMEYTSPKNQIVLKYEKQELIVLNIRNTETGDYLTLDDLAELDAENPEHTIYTHIAERFVDYEEVDGMSDEDVERIRDMKGIEGYVLVGQNQRVKLKTDWYVNLHRLKDNINNNRRLVESVVESRTDDLRQLFEHDQGSIDKIKEFEQYVLSKIKSCLAEVRTVYERVKHLDRKHYAINAQRYVDYTPLFSVIMRQFDDYNEENVVENIKQIALKNVDDFIPMHYK

SEQ ID NO: 17 - protein, 339 aa, Klebsiella phage KP27
MFKKYSSLTNHYEGKFINGVIMNGLTGGVWVAREKIHGANFSFITDDGITVTPAKRTDVVKPAEDFYGCSAVVAKYSPGIRKMWETLKKTGTYDDLVIQVYGEFAGRGVQKDVDYGEKDFYVFDIRVNGEFLPDNLCSLISRSHGLKMAPLLGYGTFEEIKELPITFESVVNKANSGIGSDNTVYGEFVYPIMDVEEGNIAEGFVMKPVSPAFMPNGERVAIKCKTTKFTEKKAKKATRFNAPVSLSEKDKNQLDEFVCYLTENRVKNVLSKLDLASITAKDFGRIMGLTVQDAIEEISRNHGPFLEQFEDPAMAKKLFVTEAQNMIRPVWGKILNHEF

SEQ ID NO: 18 - protein, 381 aa, Vibrio phage
MNVQELYKNLMSLADDAEGKFFFADHLSPLGEKFRVFSYHIASYSDWLLPGALEARGIMFQLDDNDEMIRIVSRPMEKFFNLNENPFTMELDLTTTVQLMDKADGSLISTYLSGENFALKSKTSIFSEQAVAANRYIKKPENRDLWEFCDDCTQAGLTVNMEWCAPNNRIVLEYPEAKLVILNIRDNETGDYVSFDDIPQSALMRVKQWLVDEYDPATAHEPDFVEKLRDTKGIEGMILRLANGQSVKIKTQWYVDLHSQKDSVNVPKKLVTTILNGNHDDLYALFADDKPTIERIREFDSHVTKTLTNSFNAVRQFYARNRHLARKDYAIAGQKVLKPWEFGVAMIAYQKQTVEGVYESLVTAYLKRPELAIPEKYLNGV

SEQ ID NO: 19 - protein, 335 aa, Vibrio phage JN02
MFKKYSSLENHYNSKFIEKLYTNGLTTGVWVAREKIHGTNFSLIIERDNVTCAKRTGPILPAEDFYGYEIVLKKYDKAIKAVQEVMESISTSVPVSYQVFGEFAGGGIQKGVDYGEKDFYVFDIIINTESDDTYYMSDYEMQDFCNTFGFKMAPMLGRGTFDSLIMIPNDLDSVLAAYNSTASEDLVEANNCVFDANVIGDNTAEGYVLKPCFPKWLSNGTRVAIKCKNSKFSEKKKSDKPVKTQVPLTEIDKNLLDVLACYVTLNRVNNVISKIGTVTPKDFGKVMGLTVQDILEETSREGIVLTSSDNPNLVKKELVRMVQDVLRPAWIELVS

SEQ ID NO: 20 - protein, 334 aa, Vibrio phage JS98
MFKKYSSLENHYNSKFIEKLRTNGLTGGEWVAREKIHGTNFSLIIERDAVTCAKRTGPILPAEDFYGYEIVLKNYADSIKSVQHLIESINYQSYQIYGELAGPGIQKNVDYGDKDFYVFDIRVTKEDGTESVLTDTLMEAFCIIHKFKVAPCLATGSFEDLIKLPNDFDSVIPDYNFAVDNAGLTIANSTDFIPKVEGKVFTAEGFVLKPDIPTWLPNGNRVAIKCKNSKFSEKKKSDKPIKAAVVLSQDDMDLMWQFTDYVTVNRINNVISKIGEVSKKDFGKVMGLTVQDILEEAAREELELTDAENPVEVKKQLVECVKDTLRAVWIELVS

SEQ ID NO: 21 - protein, 379 aa, Vibrio phage nt-1
MNELYNNLMTLAESAEGKFFFADHLSPQGEKFRVFSYHIASYSDWLLPDALEARGIMFQLDENDEMIRIVSRPMEKFFNLGENPFTMDLDLTTTVQLMDKADGSLISTYLTGDNFALKSKTSIYSEQAVAANRYIKHVDNRDLWEFCDDCAAQNFTVNMEWCAPNNRIVLEYTEPKLIILNIRDNETGQYVSFDDIPIGALTRIKKWLVDEYDPMTAHVDDFVETLKAKKGIEGMILRLASGQSVKIKTTWYVDLHAQKDSVNSPKKLVTTILNKNHDDLYALFADDKPTIERIREFDDHVSKKVVESFHAVSQYYTKNRHLSRKDFAIAGQKALKPWEFGVAMIAYQNQTVEGVVTMLINAYLKRPELLIPEKYLSEV

SEQ ID NO: 22 - protein, 335 aa, Vibrio phage phi-ST2
MSFVKYTSLENSYRQAFVDKCDMLGVKEWVALEKIHGANFSFIVEFKPSTEEVPGEMSVTPAKRTSTIGANAMGDYDFYGCTSVVEAHIEKMQDISNWLFANDFIKNDETIIVYGELAGKGIQKEVNYGDKDFWAYDILCPETGEFLDWDVVLKACKFAGVKTTHEIARGTLDELLKIDPLFRSFHTPADVDSENVAEGFVVKQLKAEKRLHNGSRAILKVKNEKFKEKKNKQGKTPRAKVVLTEEQEKLHAAFSCYLTENRLRNVLSKIGKVEAKQFGMVSGLFVKDAKDEFERDERDEVAIPRDDWDVIKRSLVNVANEILRKNWLNIVDGTF

SEQ ID NO: 23 - RNA, 13 nt, synthetic construct
  source 1..13: mol_type = other RNA; note; note (original language) = 底物1
tccttagtcagta

SEQ ID NO: 24 - RNA, 10 nt, synthetic construct
  source 1..10: mol_type = other RNA; note; note (original language) = 底物2
gatattttat

SEQ ID NO: 25 - RNA, 10 nt, synthetic construct
  source 1..10: mol_type = other RNA; note; note (original language) = 底物4
gactgcacta

SEQ ID NO: 26 - RNA, 50 nt, synthetic construct
  source 1..50: mol_type = other RNA; note; note (original language) = 底物5
gactgatatacacaggccgatgtggttttagagctagaaatagcaagtta

SEQ ID NO: 27 - RNA, 50 nt, synthetic construct
  source 1..50: mol_type = other RNA; note; note (original language) = 底物6
aaataaggctagtccgttatcaacttgaaaaagtggcaccgagtcggtgc

SEQ ID NO: 28 - RNA, 36 nt, synthetic construct
  source 1..36: mol_type = other RNA; note; note (original language) = 底物7
gttttagagctagaaatagcaagttaaaataaggct

SEQ ID NO: 29 - RNA, 40 nt, synthetic construct
  source 1..40: mol_type = other RNA; note; note (original language) = 底物8
agtccgttatcaacttgaaaaagtggcaccgagtcggtgc

SEQ ID NO: 30 - RNA, 10 nt, synthetic construct
  source 1..10: mol_type = other RNA; note; note (original language) = 底物11
gactgcacta